European Patent Application EP 4 763 222 A1, published June 24, 2026. Title: A Composition Comprising Apitegromab and Variants thereof, and Related Methods and Uses. Applicant: QILU PHARMACEUTICAL CO., LTD. The sequence listing filed with the application follows.

SEQUENCE LISTING (4 sequences)

SEQ ID NO: 1 - protein, 452 aa, synthetic construct
QVQLVESGGGVVQPGRSLRLSCAASGFTFSSYGMHWVRQAPGKGLEWVAVISYDGSNKYYADSVKGRFTISRDNSKNTLYLQMNSLRAEDTAVYYCARDLLVRFLEWSHYYGMDVWGQGTTVTVSSASTKGPSVFPLAPCSRSTSESTAALGCLVKDYFPEPVTVSWNSGALTSGVHTFPAVLQSSGLYSLSSVVTVPSSSLGTKTYTCNVDHKPSNTKVDKRVESKYGPPCPPCPAPEFLGGPSVFLFPPKPKDTLMISRTPEVTCVVVDVSQEDPEVQFNWYVDGVEVHNAKTKPREEQFNSTYRVVSVLTVLHQDWLNGKEYKCKVSNKGLPSSIEKTISKAKGQPREPQVYTLPPSQEEMTKNQVSLTCLVKGFYPSDIAVEWESNGQPENNYKTTPPVLDSDGSFFLYSRLTVDKSRWQEGNVFSCSVMHEALHNHYTQKSLSLSLG

SEQ ID NO: 2 - protein, 215 aa, synthetic construct
QSVLTQPPSASGTPGQRVTISCSGSSSNIGSNTVHWYQQLPGTAPKLLIYSDNQRPSGVPDRFSGSKSGTSASLAISGLQSEDEADYYCAAWDDSLNGVFGGGTKLTVLGQPKAAPSVTLFPPSSEELQANKATLVCLISDFYPGAVTVAWKADSSPVKAGVETTTPSKQSNNKYAASSYLSLTPEQWKSHRSYSCQVTHEGSTVEKTVAPTECS

SEQ ID NO: 3 - protein, 17 aa, synthetic construct
DLLVRFLEWSHYYGMDV

SEQ ID NO: 4 - protein, 27 aa, synthetic construct
FLEWSHYYGMDVWGQGTTVTVSSASTK